European Patent Application EP 4 793 283 A1, published August 19, 2026. Title: Peptides blocking amyloid fibril growth. Applicant: Ustav organicke chemie a biochemie AV CR, v. v. i. Application EP. The sequence listing filed with the application follows.

SEQUENCE LISTING (19 sequences)

SEQ ID NO: 1 - protein, 21 aa, Synthetic construct
  VARIANT 1: note = 0 to 6 amino acids, any amino acids
  VARIANT 3: note = 0 to 2 amino acids, any amino acids
  VARIANT 4: note = V or I or A or T
  VARIANT 5: note = V or I or A or T
  VARIANT 6: note = V or I or A or T
  VARIANT 7: note = V or I or A or T
  VARIANT 8: note = V or I or A or T
  VARIANT 9: note = 0 to 2 amino acids, any amino acids
  VARIANT 13: note = 0 to 2 amino acids, any amino acids
  VARIANT 14: note = V or I or A or T
  VARIANT 15: note = V or I or A or T
  VARIANT 16: note = V or I or A or T
  VARIANT 17: note = V or I or A or T
  VARIANT 18: note = V or I or A or T
  VARIANT 19: note = 0 to 2 amino acids, any amino acids
  VARIANT 21: note = 0 to 6 amino acids, any amino acids
  MOD_RES 1: note = substitution by carboxyfluorescein residue, Ph3C-CH2-CO-, Ph3P+(CH2)3-CO-, Ph2N-(C6H4)-CO- or sulforhodamine residue
XCXXXXXXXKKKXXXXXXXCX

SEQ ID NO: 2 - protein, 21 aa, Synthetic construct
  VARIANT 1: note = 0 to 6 amino acids, any amino acids
  VARIANT 3: note = 0 to 2 amino acids, any amino acids
  VARIANT 9: note = 0 to 2 amino acids, any amino acids
  VARIANT 13: note = 0 to 2 amino acids, any amino acids
  VARIANT 19: note = 0 to 2 amino acids, any amino acids
  VARIANT 21: note = 0 to 6 amino acids, any amino acids
  MOD_RES 1: note = substituted by carboxyfluorescein residue, Ph3C-CH2-CO-, Ph3P+(CH2)3-CO-, Ph2N-(C6H4)-CO- or sulforhodamine residue
XCXVATVAXKKKXVATVAXCX

SEQ ID NO: 3 - protein, 23 aa, Synthetic construct
  MOD_RES 1: note = substituted by carboxyfluorescein residue, Ph3C-CH2-CO-, Ph3P+(CH2)3-CO-, Ph2N-(C6H4)-CO- or sulforhodamine residue
KCKVATVAKKKWGVATVAKCRRK

SEQ ID NO: 4 - protein, 5 aa, Synthetic construct
VATVA

SEQ ID NO: 5 - protein, 5 aa, Synthetic construct
  VARIANT 4: note = W or H
KKKXG

SEQ ID NO: 6 - protein, 23 aa, Synthetic construct
  MOD_RES 1: note = substituted by carboxyfluorescein residue
KCKVATVAKKKWGVATVAKCRRK

SEQ ID NO: 7 - protein, 5 aa, Synthetic construct
IATIA

SEQ ID NO: 8 - protein, 5 aa, Synthetic construct
VAVVA

SEQ ID NO: 9 - protein, 23 aa, Synthetic construct
  MOD_RES 1: note = substituted by carboxyfluorescein residue
KCKVAVVAKKKWGVAVVAKCRRK

SEQ ID NO: 10 - protein, 23 aa, Synthetic construct
  MOD_RES 1: note = substituted by carboxyfluorescein residue
KCKAVTAVKKKWGAVTAVKCRRK

SEQ ID NO: 11 - protein, 23 aa, Synthetic construct
  MOD_RES 1: note = substituted by carboxyfluorescein residue
KCKIATIAKKKWGIATIAKCRRK

SEQ ID NO: 12 - protein, 21 aa, Synthetic construct
  MOD_RES 1: note = substituted by carboxyfluorescein residue
KCKVATVAKKKVATVAKCRRK

SEQ ID NO: 13 - protein, 23 aa, Synthetic construct
  MOD_RES 1: note = substituted by Ph3C-CH2-CO
KCKVATVAKKKWGVATVAKCRRK

SEQ ID NO: 14 - protein, 23 aa, Synthetic construct
  MOD_RES 14: note = substituted by Ph3P+CH2CH2CH2CO
KCKVATVAKKKWGVATVAKCRRK

SEQ ID NO: 15 - protein, 21 aa, Synthetic construct
  MOD_RES 1: note = acylation
WGKCVATVAKKKHGVATVACE

SEQ ID NO: 16 - protein, 20 aa, Synthetic construct
  MOD_RES 1: note = substituted by carboxyfluorescein residue
GKCVATVAKKKHGVATVACE

SEQ ID NO: 17 - protein, 20 aa, Synthetic construct
  MOD_RES 1: note = substituted by carboxyfluorescein residue
GKCVATVAKKKHGVATVACE

SEQ ID NO: 18 - protein, 19 aa, Synthetic construct
  MOD_RES 1: note = substituted by carboxyfluorescein residue
GKGVATVAKKKHGVATVAE

SEQ ID NO: 19 - protein, 4 aa, Synthetic construct
KRRK